European Patent Specification EP 3 436 591 B1, published January 4, 2023. Title: Adenoviral Coat Protein Derived Delivery Vehicles. Applicant: European Molecular Biology Laboratory. The sequence listing filed with the application follows.

SEQUENCE LISTING (78 sequences)

SEQ ID NO: 1 - protein, 544 aa, Adenovirus type B 3
MRRRAVLGGAVVYPEGPPPSYESVMQQQAAMIQPPLEAPFVPPRYLAPTEGRNSIRYSELSPLYDTTKLYLVDNKSADIASLNYQNDHSNFLTTVVQNNDFTPTEASTQTINFDERSRWGGQLKTIMHTNMPNVNEYMFSNKFKARVMVSRKAPEGVTVNDTYDHKEDILKYEWFEFILPEGNFSATMTIDLMNNAIIDNYLEIGRQNGVLESDIGVKFDTRNFRLGWDPETKLIMPGVYTYEAFHPDIVLLPGCGVDFTESRLSNLLGIRKRHPFQEGFKIMYEDLEGGNIPALLDVTAYEESKKDTTTETTTLAVAEETSEDDDITRGDTYITEKQKREAAAAEVKKELKIQPLEKDSKSRSYNVLEDKINTAYRSWYLSYNYGNPEKGIRSWTLLTTSDVTCGAEQVYWSLPDMMQDPVTFRSTRQVNNYPVVGAELMPVFSKSFYNEQAVYSQQLRQATSLTHVFNRFPENQILIRPPAPTITTVSENVPALTDHGTLPLRSSIRGVQRVTVTDARRRTCPYVYKALGIVAPRVLSSRTF

SEQ ID NO: 2 - protein, 571 aa, Adenovirus type C 2
MQRAAMYEEGPPPSYESVVSAAPVAAALGSPFDAPLDPPFVPPRYLRPTGGRNSIRYSELAPLFDTTRVYLVDNKSTDVASLNYQNDHSNFLTTVIQNNDYSPGEASTQTINLDDRSHWGGDLKTILHTNMPNVNEFMFTNKFKARVMVSRSLTKDKQVELKYEWVEFTLPEGNYSETMTIDLMNNAIVEHYLKVGRQNGVLESDIGVKFDTRNFRLGFDPVTGLVMPGVYTNEAFHPDIILLPGCGVDFTHSRLSNLLGIRKRQPFQEGFRITYDDLEGGNIPALLDVDAYQASLKDDTEQGGDGAGGGNNSGSGAEENSNAAAAAMQPVEDMNDHAIRGDTFATRAEEKRAEAEAAAEAAAPAAQPEVEKPQKKPVIKPLTEDSKKRSYNLISNDSTFTQYRSWYLAYNYGDPQTGIRSWTLLCTPDVTCGSEQVYWSLPDMMQDPVTFRSTSQISNFPVVGAELLPVHSKSFYNDQAVYSQLIRQFTSLTHVFNRFPENQILARPPAPTITTVSENVPALTDHGTLPLRNSIGGVQRVTITDARRRTCPYVYKALGIVSPRVLSSRTF

SEQ ID NO: 3 - protein, 561 aa, Adenovirus type B 35
MRRVVLGGAVVYPEGPPPSYESVMQQQQATAVMQSPLEAPFVPPRYLAPTEGRNSIRYSELAPQYDTTRLYLVDNKSADIASLNYQNDHSNFLTTVVQNNDFTPTEASTQTINFDERSRWGGQLKTIMHTNMPNVNEYMFSNKFKARVMVSRKPPDGAAVGDTYDHKQDILEYEWFEFTLPEGNFSVTMTIDLMNNAIIDNYLKVGRQNGVLESDIGVKFDTRNFKLGWDPETKLIMPGVYTYEAFHPDIVLLPGCGVDFTESRLSNLLGIRKKQPFQEGFKILYEDLEGGNIPALLDVDAYENSKKEQKAKIEAATAAAEAKANIVASDSTRVANAGEVRGDNFAPTPVPTAESLLADVSEGTDVKLTIQPVEKDSKNRSYNVLEDKINTAYRSWYLSYNYGDPEKGVRSWTLLTTSDVTCGAEQVYWSLPDMMKDPVTFRSTRQVSNYPVVGAELMPVFSKSFYNEQAVYSQQLRQSTSLTHVFNRFPENQILIRPPAPTITTVSENVPALTDHGTLPLRSSIRGVQRVTVTDARRRTCPYVYKALGIVAPRVLSSRTF

SEQ ID NO: 4 - protein, 535 aa, Adenovirus type E 4
MMRRAYPEGPPPSYESVMQQAMAAAAAIQPPLEAPYVPPRYLAPTEGRNSIRYSELTPLYDTTRLYLVDNKSADIASLNYQNDHSNFLTTVVQNNDFTPTEASTQTINFDERSRWGGQLKTIMHTNMPNVNQFMYSNKFKARVMVSRKTPNGVTVGDNYDGSQDELKYEWVEFELPEGNFSVTMTIDLMNNAIIDNYLAVGRQNGVLESDIGVKFDTRNFRLGWDPVTELVMPGVYTNEAFHPDIVLLPGCGVDFTESRLSNLLGIRKRQPFQEGFQIMYEDLDGGNIPALLDVEAYEKSKEESVAAATTAVATASTEVRDDNFASAAAVAAVKADETKSKIVIQPVEKDSKERSYNVLSDKKNTAYRSWYLAYNYGDRDKGVRSWTLLTTSDVTCGVEQVYWSLPDMMQDPVTFRSTHQVSNYPVVGAELLPVYSKSFFNEQAVYSQQLRAFTSLTHVFNRFPENQILVRPPAPTITTVSENVPALTDHGTLPLRSSIRGVQRVTVTDARRRTCPYVYKALGIVAPRVLSSRTF

SEQ ID NO: 5 - protein, 571 aa, Adenovirus type C 5
MRRAAMYEEGPPPSYESVVSAAPVAAALGSPFDAPLDPPFVPPRYLRPTGGRNSIRYSELAPLFDTTRVYLVDNKSTDVASLNYQNDHSNFLTTVIQNNDYSPGEASTQTINLDDRSHWGGDLKTILHTNMPNVNEFMFTNKFKARVMVSRLPTKDNQVELKYEWVEFTLPEGNYSETMTIDLMNNAIVEHYLKVGRQNGVLESDIGVKFDTRNFRLGFDPVTGLVMPGVYTNEAFHPDIILLPGCGVDFTHSRLSNLLGIRKRQPFQEGFRITYDDLEGGNIPALLDVDAYQASLKDDTEQGGGGAGGSNSSGSGAEENSNAAAAAMQPVEDMNDHAIRGDTFATRAEEKRAEAEAAAEAAAPAAQPEVEKPQKKPVIKPLTEDSKKRSYNLISNDSTFTQYRSWYLAYNYGDPQTGIRSWTLLCTPDVTCGSEQVYWSLPDMMQDPVTFRSTRQISNFPVVGAELLPVHSKSFYNDQAVYSQLIRQFTSLTHVFNRFPENQILARPPAPTITTVSENVPALTDHGTLPLRNSIGGVQRVTITDARRRTCPYVYKALGIVSPRVLSSRTF

SEQ ID NO: 6 - protein, 532 aa, Adenovirus type Y25
MMRRAYPEGPPPSYESVMQQAMAAAAAMQPPLEAPYVPPRYLAPTEGRNSIRYSELAPLYDTTRLYLVDNKSADIASLNYQNDHSNFLTTVVQNNDFTPTEASTQTINFDERSRWGGQLKTIMHTNMPNVNEFMYSNKFKARVMVSRKTPNGVTVTDGSQDILEYEWVEFELPEGNFSVTMTIDLMNNAIIDNYLAVGRQNGVLESDIGVKFDTRNFRLGWDPVTELVMPGVYTNEAFHPDIVLLPGCGVDFTESRLSNLLGIRKRQPFQEGFQIMYEDLEGGNIPALLDVDAYEKSKEESAAAATAAVATASTEVRGDNFASPAAVAAAEAAETESKIVIQPVEKDSKDRSYNVLPDKINTAYRSWYLAYNYGDPEKGVRSWTLLTTSDVTCGVEQVYWSLPDMMQDPVTFRSTRQVSNYPVVGAELLPVYSKSFFNEQAVYSQQLRAFTSLTHVFNRFPENQILVRPPAPTITTVSENVPALTDHGTLPLRSSIRGVQRVTVTDARRRTCPYVYKALGIVAPRVLSSRTF

SEQ ID NO: 7 - protein, 575 aa, Adenovirus type B 7
MMRRAVLGGAVVYPEGPPPSYESVMQQQAAAVMQPSLEAPFVPPRYLAPTEGRNSIRYSELAPQYDTTRLYLVDNKSADIASLNYQNDHSNFLTTVVQNNDFTPTEASTQTINFDERSRWGGQLKTIMHTNMPNVNEYMFSNKFKARVMVSREASKIDSEKNDRSKDTLKYEWFEFTLPEGNFSATMTIDLMNNAIIDNYLAVGRQNGVLQSDIGVKFDTRNFRLGWDPVTKLVMPGVYTYEAFHPDIVLLPDCGVDFTESRLSNLLGIRKRHPFQEGFKIMYEDLEGGNIPALLDVAEYEKSKKEIASSTTTTAVTTVARNVADTSVEAVAVAVVDTIKAENDSAVRGDNFQSKNDMKASEEVTVVPVSPPTVTETETKEPTIKPLEKDTKDRSYNVISGTNDTAYRSWYLAYNYGDPEKGVRSWTLLTTSDVTCGAEQVYWSLPDMMQDPVTFRSTRQVSNYPVVGAELMPVFSKSFYNEQAVYSQQLRQTTSLTHIFDRFPENQILIRPPAPTITTVSENVPALTDHGTLPLRSSIRGVQRVTVTDARRRTCPYVYKALGIVAPRVLSSRTF

SEQ ID NO: 8 - protein, 503 aa, Adenovirus type 52
MRRAVRVTPAAYEGPPPSYESVMGSANVPATLEAPYVPPRYLGPTEGRNSIRYSELAPLYDTTKVYLVDNKSADIASLNYQNDHSNFLTTVVQNNDFTPTEAGTQTINFDERSRWGGQLKTILHTNMPNINEFMSTNKFRARLMVKKVENQPPEYEWFEFTIPEGNYSETMTIDLMNNAIVDNYLQVGRQNGVLESDIGVKFDTRNFRLGWDPVTKLVMPGVYTNEAFHPDIVLLPGCGVDFTQSRLSNLLGIRKRRPFQEGFQIMYEDLEGGNIPALLDVTKYEQSVQRAKAEGREIRGDTFAVSPQDLVIEPLEHDSKNRSYNLLPNKTDTAYRSWFLAYNYGDPEKGVRSWTILTTTDVTCGSQQVYWSLPDMMQDPVTFRPSTQVSNFPVVGTELLPVHAKSFYNEQAVYSQLIRQSTALTHVFNRFPENQILVRPPAPTITTVSENVPALTDHGTLPLRSSISGVQRVTITDARRRTCPYVYKALGVVAPKVLSSRTF

SEQ ID NO: 9 - protein, 504 aa, Adenovirus type 53
MRRAVRVTPAVYAEGPPPSYESVMGSANVPATLEAPYVPPRYLGPTEGRNSIRYSELAPLYDTTKVYLVDNKSADIASLNYQNDHSNFLTTVVQNNDFTPTEAGTQTINFDERSRWGGQLKTILHTNMPNINEFMSTNKFRARLMVEKTSGQPPKYEWFEFTIPEGNYSETMTIDLMNNAIVDNYLQVGRQNGVLESDIGVKFDTRNFRLGWDPVTKLVMPGVYTNEAFHPDIVLLPGCGVDFTQSRLSNLLGIRKRRPFQEGFQIMYEDLEGGNIPGLLDVPAYEQSLQQAQEEGRVTRGDTFATAPNEVVIKPLLKDSKDRSYNIITDTTDTLYRSWFLAYNYGDPENGVRSWTILTTTDVTCGSQQVYWSLPDMMQDPVTFRPSTQVSNFPVVGTELLPVHAKSFYNEQAVYSQLIRQSTALTHVFNRFPENQILVRPPAPTITTVSENVPALTDHGTLPLRSSISGVQRVTITDARRRTCPYVYKALGVVAPKVLSSRTF

SEQ ID NO: 10 - protein, 505 aa, Adenovirus type 51
MRRAVRVTPAAYEGPPPSYESVMGSANVPATLEAPYVPPRYLGPTEGRNSIRYSELAPLYDTTKVYLVDNKSADIASLNYQNDHSNFLTTVVQNNDFTPTEAGTQTINFDERSRWGGQLKTILHTNMPNINEFMSTNKFRAKLMVEKSNAETRQPRYEWFEFTIPEGNYSETMTIDLMNNAIVDNYLQVGRQNGVLESDIGVKFDTRNFRLGWDPVTKLVMPGVYTNEAFHPDIVLLPGCGVDFTQSRLSNLLGIRKRRPFQEGFQIMYEDLEGGNIPALLDVSKYEASIQRAKAEGREIRGDTFAVAPQDLEIVPLTKDSKDRSYNIINNTTDTLYRSWFLAYNYGDPEKGVRSWTILTTTDVTCGSQQVYWSLPDMMQDPVTFRPSTQVSNFPVVGTELLPVHAKSFYNEQAVYSQLIRQSTALTHVFNRFPENQILVRPPAPTITTVSENVPALTDHGTLPLRSSISGVQRVTITDARRRTCPYVYKALGVVAPKVLSSRTF

SEQ ID NO: 11 - protein, 508 aa, Adenovirus type 18
MRRAVGVPPVMAYAEGPPPSYETVMGAADSPATLEALYVPPRYLGPTEGRNSIRYSELAPLYDTTRVYLVDNKSADIASLNYQNDHSNFLTTVVQNNDFTPVEAGTQTINFDERSRWGGDLKTILRTNMPNINEFMSTNKFRARLMVEKVNKETNAPRYEWFEFTLPEGNYSETMTIDLMNNAIVDNYLEVGRQNGVLESDIGVKFDTRNFRLGWDPVTKLVMPGVYTNEAFHPDIVLLPGCGVDFTQSRLSNLLGIRKRMPFQAGFQIMYEDLEGGNIPALLDVAKYEASIQKAREQGQEIRGDNFTVIPRDVEIVPVEKDSKDRSYNLLPGDQTNTAYRSWFLAYNYGDPEKGVRSWTLLTTTDVTCGSQQVYWSLPDMMQDPVTFRPSSQVSNYPVVGVELLPVHAKSFYNEQAVYSQLIRQSTALTHVFNRFPENQILVRPPAPTITTVSENVPALTDHGTLPLRSSISGVQRVTITDARRRTCPYVHKALGIVAPKVLSSRTF

SEQ ID NO: 12 - protein, 511 aa, Adenovirus type 49
MRRAVPAAAIPATVAYADPPPSYESVMAGVPATLEAPYVPPRYLGPTEGRNSIRYSELAPLYDTTRVYLVDNKSADIASLNYQNDHSNFLTTVVQNNDFTPVEAGTQTINFDERSRWGGQLKTILHTNMPNVNEFMFTNSFRAKVMVSRKQNEEGQTELEYEWVEFVLPEGNYSETMTLDLMNNAIVDHYLLVGRQNGVLESDIGVKFDTRNFRLGWDPVTKLVMPGVYTNEAFHPDVVLLPGCGVDFTQSRLSNLLGIRKRQPFQEGFRIMYEDLEGGNIPALLNVKAYEDSIAAAMRKHNLPLRGDVFAVQPQEIVIQPVEKDGKERSYNLLPDDKNNTAYRSWYLAYNYGDPLKGVRSWTLLTTPDVTCGSEQVYWSLPDLMQDPVTFRPSSQVSNYPVVGAELLPLQAKSFYNEQAVYSQLIRQSTALTHVFNRFPENQILVRPPAATITTVSENVPALTDHGTLPLRSSISGVQRVTITDARRRTCPYVYKALGIVAPRVLSSRTF

SEQ ID NO: 13 - protein, 512 aa, Adenovirus type 20
MRRAVAIPSAAVALGPPPSYESVMASANLQAPLENPYVPPRYLEPTGGRNSIRYSELTPLYDTTRLYLVDNKSADIATLNYQNDHSNFLTSVVQNSDYTPAEASTQTINLDDRSRWGGDLKTILHTNMPNVNEFMFTNSFRAKLMVAHETNKDPVYKWVELTLPEGNFSETMTIDLMNNAIVDHYLAVGRQNGVKESEIGVKFDTRNFRLGWDPQTELVMPGVYTNEAFHPDVVLLPGCGVDFTYSRLSNLLGIRKRMPFQEGFQIMYEDLVGGNIPALLDVPAYEASITTVAAKEVRGDNFEAAAAAAATGAQPQAAPVVRPVTQDSKGRSYNIITGTNNTAYRSWYLAYNYGDPEKGVRSWTLLTTPDVTCGSEQVYWSMPDMYVDPVTFRSSQQVSSYPVVGAELLPIHSKSFYNEQAVYSQLIRQQTALTHVFNRFPENQILVRPPAPTITTVSENVPALTDHGTLPLQNSIRGVQRVTITDARRRTCPYVYKALGIVAPRVLSSRTF

SEQ ID NO: 14 - protein, 497 aa, Adenovirus type 12
MRRAVELQTVAFPETPPPSYETVMAAAPPYVPPRYLGPTEGRNSIRYSELSPLYDTTRVYLVDNKSSDIASLNYQNDHSNFLTTVVQNNDYSPIEAGTQTINFDERSRWGGDLKTILHTNMPNVNDFMFTTKFKARVMVARKTNNEGQTILEYEWAEFVLPEGNYSETMTIDLMNNAIIEHYLRVGRQHGVLESDIGVKFDTRNFRLGWDPETQLVTPGVYTNEAFHPDIVLLPGCGVDFTESRLSNILGIRKRQPFQEGFVIMYEHLEGGNIPALLDVKKYENSLQDQNTVRGDNFIALNKAARIEPVETDPKGRSYNLLPDKKNTKYRSWYLAYNYGDPEKGVRSWTLLTTPDVTGGSEQVYWSLPDMMQDPVTFRSSRQVSNYPVVAAELLPVHAKSFYNEQAVYSQLIRQSTALTRVFNRFPENQILVRPPAATITTVSENVPALTDHGTLPLRSSISGVQRVTITDARRRTCPYVYKALGIVSPRVLSSRTF

SEQ ID NO: 15 - protein, 9 aa, Artificial Sequence
  Consensus sequence of penton base proteins
  MISC_FEATURE (1)..(1): Xaa is selected from the group consisting of D, E and N, and is preferably D
  MISC_FEATURE (2)..(2): is selected from the group consisting of V, L, and I, and is preferably V
  MISC_FEATURE (3)..(3): is any amino acid, is preferably selected from the group consisting of A, D, E, K, S, and T, and is more preferably T
  MISC_FEATURE (4)..(4): is any amino acid, is preferably selected from the group consisting of A, D, E, and K, and is more preferably A
  MISC_FEATURE (5)..(5): is selected from the group consisting of F, Y, and W, and is preferably Y
  MISC_FEATURE (6)..(6): is selected from the group consisting of A, D, E, N, and Q, is preferably E or Q, and is more preferably E
  MISC_FEATURE (7)..(7): is any amino acid, preferably selected from the group consisting of A, D, E, N, and K, and is more preferably E
  MISC_FEATURE (8)..(8): is selected from the group consisting of S or T, and is preferably S
  MISC_FEATURE (9)..(9): is any amino acid
XXXXXXXXX

SEQ ID NO: 16 - protein, 5 aa, Artificial Sequence
  Consensus sequence of penton base proteins
  MISC_FEATURE (1)..(1): is any amino acid
  MISC_FEATURE (2)..(2): is R
  MISC_FEATURE (3)..(3): is G
  MISC_FEATURE (4)..(4): is D
  MISC_FEATURE (5)..(5): is any amino acid
XXXXX

SEQ ID NO: 17 - protein, 8 aa, Artificial Sequence
  Consensus sequence of penton base proteins
  MISC_FEATURE (1)..(1): is any amino acid
  MISC_FEATURE (2)..(2): is selected from the group consisting of I, L and V, and is preferably I
  MISC_FEATURE (3)..(3): is selected from the group consisting of D, E, K, N, Q, and V, is preferably Q or K, and is more preferably Q
  MISC_FEATURE (4)..(4): is selected from the group consisting of C, G and P, and is preferably P
  MISC_FEATURE (5)..(5): is selected from the group consisting of I, L and V, is preferably L or V and is more preferably L
  MISC_FEATURE (6)..(6): is selected from the group consisting of D, E, S and T, is preferably E or T and is more preferably E
  MISC_FEATURE (7)..(7): is selected from the group consisting of D, E, K, S and T, is preferably E, K or T, and is more preferably K
  MISC_FEATURE (8)..(8): is selected from the group consisting of D and E, and is preferably D
XXXXXXXX

SEQ ID NO: 18 - protein, 8 aa, Artificial Sequence
  Consensus sequence of penton base proteins
  MISC_FEATURE (1)..(1): is selected from the group consisting of F, Y, and W, and is preferably F
  MISC_FEATURE (2)..(2): is selected from the group consisting of H, K and R, and is preferably K
  MISC_FEATURE (3)..(3): is selected from the group consisting of A, V, I, and L, and is preferably A
  MISC_FEATURE (4)..(4): is selected from the group consisting of H, K, and R, and is preferably R
  MISC_FEATURE (5)..(5): is selected from the group consisting of A, V, I, and L, and is preferably V
  MISC_FEATURE (6)..(6): is selected from the group consisting of A, V, I, L and M, and is preferably M
  MISC_FEATURE (7)..(7): is selected from the group consisting of A, V, I, and L, and is preferably V
  MISC_FEATURE (8)..(8): is any amino acid
XXXXXXXX

SEQ ID NO: 19 - protein, 7 aa, Artificial Sequence
  Consensus sequence of penton base proteins
  MISC_FEATURE (1)..(1): is any amino acid
  MISC_FEATURE (2)..(2): is selected from the group consisting of F, Y, and W, and is preferably Y
  MISC_FEATURE (3)..(3): is selected from the group consisting of D, E, S and T, is preferably E or T and is more preferably E
  MISC_FEATURE (4)..(4): is selected from the group consisting of F, Y, and W, and is preferably W
  MISC_FEATURE (5)..(5): is selected from the group consisting of A, F, V, Y, and W, is preferably F or V and is more preferably F
  MISC_FEATURE (6)..(6): is selected from the group consisting of D, E, S and T, is preferably D or E and is more preferably E
  MISC_FEATURE (7)..(7): is selected from the group consisting of F, Y, and W, and is preferably F
XXXXXXX

SEQ ID NO: 20 - protein, 26 aa, Artificial Sequence
  Consensus sequence of peton base proteins
  MISC_FEATURE (11)..(11): Xaa is selected from the group consisting of V, I, and L
  MISC_FEATURE (12)..(12): Xaa is selected from the group consisting of E, and D
  MISC_FEATURE (13)..(13): Xaa is selected from the group consisting of H, N and Q
  MISC_FEATURE (16)..(16): Xaa is selected from the group consisting of K, E, R, Q, and A
  MISC_FEATURE (17)..(17): Xaa is selected from the group consisting of V, L, and I
  MISC_FEATURE (21)..(21): Xaa is selected from the group consisting of H, N and Q
MTIDLMNNAIXXXYLXXGRQXGVLES

SEQ ID NO: 21 - protein, 8 aa, Adenovirus
DVTAYEES

SEQ ID NO: 22 - protein, 8 aa, Adenovirus
DVDAYENS

SEQ ID NO: 23 - protein, 8 aa, Adenovirus
DVAEYEKS

SEQ ID NO: 24 - protein, 8 aa, Adenovirus
DVEAYEKS

SEQ ID NO: 25 - protein, 8 aa, Adenovirus
DVDAYEKS

SEQ ID NO: 26 - protein, 8 aa, Adenovirus
DVSKYEAS

SEQ ID NO: 27 - protein, 8 aa, Adenovirus
NVKAYEDS

SEQ ID NO: 28 - protein, 8 aa, Adenovirus
DVKKYENS

SEQ ID NO: 29 - protein, 8 aa, Adenovirus
DVDAYQAS

SEQ ID NO: 30 - protein, 8 aa, Adenovirus
DVDAYQAS

SEQ ID NO: 31 - protein, 7 aa, Adenovirus
IQPLEKD

SEQ ID NO: 32 - protein, 7 aa, Adenovirus
IQPVEKD

SEQ ID NO: 33 - protein, 7 aa, Adenovirus
IKPLEKD

SEQ ID NO: 34 - protein, 7 aa, Adenovirus
IVPLTKD

SEQ ID NO: 35 - protein, 7 aa, Adenovirus
IEPVETD

SEQ ID NO: 36 - protein, 7 aa, Adenovirus
IKPLTED

SEQ ID NO: 37 - protein, 7 aa, Adenovirus
FKARVMV

SEQ ID NO: 38 - protein, 7 aa, Adenovirus
FRAKLMV

SEQ ID NO: 39 - protein, 7 aa, Adenovirus
FRAKVMV

SEQ ID NO: 40 - protein, 6 aa, Adenovirus
YEWFEF

SEQ ID NO: 41 - protein, 6 aa, Adenovirus
YEWVEF

SEQ ID NO: 42 - protein, 6 aa, Adenovirus
YEWAEF

SEQ ID NO: 43 - protein, 9 aa, Artificial Sequence
  Adenovirus fibre protein consensus sequence
  MISC_FEATURE (1)..(1): is selected from the group consisting of S, D and T, preferably S or D, and is more preferably S
  MISC_FEATURE (9)..(9): is selected from the group consisting of E, D and G, is preferably E or D, and is more preferably E
XFNPVYPYX

SEQ ID NO: 44 - protein, 7 aa, Artificial Sequence
  Consensus sequence of the N-terminus of the N-terminal domain
  MISC_FEATURE (1)..(1): Xaa is selected from the group consisting of G and E
XGRNSIR

SEQ ID NO: 45 - protein, 6 aa, Artificial Sequence
  C-terminalconsensus sequence of the N-terminal domain
  MISC_FEATURE (2)..(2): Xaa is selected from the group consisting of D and E
DXRSRG

SEQ ID NO: 46 - protein, 9 aa, Artificial Sequence
  Part of the conformational epitope forming the fibre binding cleft of the penton base protomer
  MISC_FEATURE (4)..(4): Xaa is selected from the group consisting of V, I, L, E, or D
  MISC_FEATURE (6)..(6): Xaa is selected from the group consisting of V, L, and I
  MISC_FEATURE (7)..(7): Xaa  is selected from the group consisting of M, T and S
WDPXTXXPG

SEQ ID NO: 47 - protein, 7 aa, Artificial Sequence
  Part of the conformational epitope forming the fibre binding cleft of the penton base protomer
  MISC_FEATURE (1)..(1): Xaa is selected from the group consisting of D, E, N, and Q
  MISC_FEATURE (3)..(3): Xaai s any amino acid, preferably selected from the group consisting of A, D, P, K and T
  MISC_FEATURE (4)..(4): Xaa is selected from the group consisting of A, D, E, K and R
  MISC_FEATURE (6)..(6): Xaais selected from the group consisting of D, E, L, I, Q, and N
  MISC_FEATURE (7)..(7): Xaa is selected from the group consisting of A, D, E, K, N, Q, and R
XVXXYXX

SEQ ID NO: 48 - protein, 5 aa, Artificial Sequence
  Part of the conformational epitope forming the fibre binding cleft of the penton base protomer
  MISC_FEATURE (1)..(1): Xaa is selected from the group consisting of K, R, S, and T
  MISC_FEATURE (2)..(2): Xaa is selected from the group consisting of A, D, E, G, K, N, Q, R, S, and T
XXRSY

SEQ ID NO: 49 - protein, 10 aa, Artificial Sequence
  Part of the conformational epitope forming the fibre binding cleft of the penton base protomer
  MISC_FEATURE (3)..(3): Xaa is selected from the group consisting of H, K, and R
  MISC_FEATURE (10)..(10): Xaa is selected from the group consisting of D and E
LTXVFNRFPX

SEQ ID NO: 50 - protein, 9 aa, Artificial Sequence
  Consensus sequence of N-terminal domain comprising coupling residues
  MISC_FEATURE (3)..(3): Xaa is selected from the group consisting of G and E
  MISC_FEATURE (4)..(4): Xaa is a coupling residue, preferably C; D, E, and K, most preferably C
  MISC_FEATURE (7)..(7): Xaa is a coupling residue, preferably C; D, E, and K, most preferably C
PTXXRNXIR

SEQ ID NO: 51 - protein, 9 aa, Artificial Sequence
  Consensus sequence of N-terminal domain comprising coupling residues
  MISC_FEATURE (3)..(3): Xaa is selected from the group consisting of G and E
  MISC_FEATURE (6)..(6): Xaa is a coupling residue, preferably C; D, E, and K, most preferably C
PTXGRXSIR

SEQ ID NO: 52 - protein, 8 aa, Artificial Sequence
  Consensus sequence of N-terminal domain comprising coupling residues
  MISC_FEATURE (6)..(6): Xaa is selected from the group consisting of D and E
  MISC_FEATURE (7)..(7): Xaa is a coupling residue, preferably C; D, E, and K, most preferably C
  MISC_FEATURE (8)..(8): Xaa is selected from the group consisting of I, L and V
TQTINXXX

SEQ ID NO: 53 - protein, 9 aa, Artificial Sequence
  Consensus sequence of N-terminal domain comprising coupling residues
  MISC_FEATURE (3)..(3): Xaa is selected from the group consisting of G and E
  MISC_FEATURE (7)..(7): Xaa is a coupling residue, preferably C; D, E, and K, most preferably C
PTXGRNXIR

SEQ ID NO: 54 - protein, 10 aa, Artificial Sequence
  Consenus sequence for the locaion of a coupling residue in the C-terminal end of the penton base protomer
  MISC_FEATURE (4)..(4): Xaa is a coupling residue, preferably C; D, E, and K, most preferably C
  MISC_FEATURE (6)..(6): Xaa is selected from the group consisting of H and Y
TCPXVXKALG

SEQ ID NO: 55 - protein, 17 aa, Dengue virus
HAKKQDVVVLGSQEGAM

SEQ ID NO: 56 - protein, 18 aa, Chikungunya virus
STKDNFNVYKATRPYLAH

SEQ ID NO: 57 - protein, 17 aa, Zika virus
STKDNFNVYKATRPLAH

SEQ ID NO: 58 - protein, 37 aa, Artificial Sequence
  Fusion protein of Chikungunya antigenic peptide and STICKER
AKRARLSTSFNPVPYEDESSTKDNFNVYKATRPYLAH

SEQ ID NO: 59 - protein, 38 aa, Artificial Sequence
  Fusion protein of STICKER with coupling residue and Chinkungunya virus antigenic peptide
AKRARLSTSFNPVPYEDECSSTKDNFNVYKATRPYLAH

SEQ ID NO: 60 - protein, 37 aa, Artificial Sequence
  Fusion protein of STICKER with coupling residue and Chinkungunya virus antigenic peptide
AKRARLSTCFNPVPYEDESSTKDNFNVYKATRPYLAH

SEQ ID NO: 61 - DNA, 4453 bp, Artificial Sequence
  Cloning vector pACEBac-ADDomer1.0 plasmid sequence
accggttgacttgggtcaactgtcagaccaagtttactcatatatactttagattgatttaaaacttcatttttaatttaaaaggatctaggtgaagatcctttttgataatctcatgaccaaaatcccttaacgtgagttttcgttccactgagcgtcagaccccgtagaaaagatcaaaggatcttcttgagatcctttttttctgcgcgtaatctgctgcttgcaaacaaaaaaaccaccgctaccagcggtggtttgtttgccggatcaagagctaccaactctttttccgaaggtaactggcttcagcagagcgcagataccaaatactgttcttctagtgtagccgtagttaggccaccacttcaagaactctgtagcaccgcctacatacctcgctctgctaatcctgttaccagtggctgctgccagtggcgataagtcgtgtcttaccgggttggactcaagacgatagttaccggataaggcgcagcggtcgggctgaacggggggttcgtgcacacagcccagcttggagcgaacgacctacaccgaactgagatacctacagcgtgagctatgagaaagcgccacgcttcccgaagggagaaaggcggacaggtatccggtaagcggcagggtcggaacaggagagcgcacgagggagcttccagggggaaacgcctggtatctttatagtcctgtcgggtttcgccacctctgacttgagcgtcgatttttgtgatgctcgtcaggggggcggagcctatggaaaaacgccagcaacgcggcctttttacggttcctggccttttgctggccttttgctcacatgttctttcctgcgttatcccctgattgacttgggtcgctcttcctgtggatgcgcagatgccctgcgtaagcgggtgtgggcggacaataaagtcttaaactgaacaaaatagatctaaactatgacaataaagtcttaaactagacagaatagttgtaaactgaaatcagtccagttatgctgtgaaaaagcatactggacttttgttatggctaaagcaaactcttcattttctgaagtgcaaattgcccgtcgtattaaagaggggcgtggccaagggcatgtaaagactatattcgcggcgttgtgacaatttaccgaacaactccgcggccgggaagccgatctcggcttgaacgaattgttaggtggcggtacttgggtcgatatcaaagtgcatcacttcttcccgtatgcccaactttgtatagagagccactgcgggatcgtcaccgtaatctgcttgcacgtagatcacataagcaccaagcgcgttggcctcatgcttgaggagattgatgagcgcggtggcaatgccctgcctccggtgctcgccggagactgcgagatcatagatatagatctcactacgcggctgctcaaacttgggcagaacgtaagccgcgagagcgccaacaaccgcttcttggtcgaaggcagcaagcgcgatgaatgtcttactacggagcaagttcccgaggtaatcggagtccggctgatgttgggagtaggtggctacgtctccgaactcacgaccgaaaagatcaagagcagcccgcatggatttgacttggtcagggccgagcctacatgtgcgaatgatgcccatacttgagccacctaactttgttttagggcgactgccctgctgcgtaacatcgttgctgctgcgtaacatcgttgctgctccataacatcaaacatcgacccacggcgtaacgcgcttgctgcttggatgcccgaggcatagactgtacaaaaaaacagtcataacaagccatgaaaaccgccactgcgccgttaccaccgctgcgttcggtcaaggttctggaccagttgcgtgagcgcatacgctacttgcattacagtttacgaaccgaacaggcttatgtcaactgggttcgtgccttcatccgtttccacggtgtgcgtcacccggcaaccttgggcagcagcgaagtcgccataacttcgtatagcatacattatacgaagttatctgtaactataacggtcctaaggtagcgagtttaaacactagtatcgattcgcgacctactccggaatattaatagatcatggagataattaaaatgataaccatctcgcaaataaataagtattttactgttttcgtaacagttttgtaataaaaaaacctataaatattccggattattcataccgtcccaccatcgggcgcggatccatgaggagacgagccgtgctaggcggagcggtggtgtatccggagggtcctcctccttcttacgagagcgtgatgcagcaacaggcggcgatgatacagcccccactggaggctcccttcgtacccccacggtacctggcgcctacggaagggagaaacagcattcgttactcggagctgtcgcccctgtacgataccaccaagttgtatctggtggacaacaagtcggcggacatcgcctccctgaactatcagaacgaccacagcaacttcctgaccacggtggtgcagaacaatgactttacccccacggaggctagcacccagaccatcaactttgacgagcggtcgcgatggggcggtcagctgaagaccatcatgcacaccaacatgcccaacgtgaacgagtacatgttcagcaacaagttcaaggcgagggtgatggtgtccagaaaagctcctgaaggtgttacagtaaatgacacctatgatcataaagaggatatcttgaagtatgagtggtttgagttcattttaccagaaggcaacttttcagccaccatgacgatcgacctgatgaacaatgccatcattgacaactacctggaaattggcagacagaatggagtgctggaaagtgacattggtgttaagtttgacactagaaatttcaggctcgggtgggaccccgaaactaagttgattatgccaggtgtctacacttatgaggcattccatcctgacattgtattgctgcctggttgcggggtagactttactgaaagccgacttagcaacttgcttggcatcaggaagagacatccattccaggagggtttcaaaatcatgtatgaagatcttgaagggggtaatattcctgcccttttggatgtcactgcctatgaggaaagcaaaaaggataccactactgaaacaaccacactggctgttgcagaggaaactagtgaagatgatgatataactagaggagatacctatataactgaaaaacaaaaacgtgaagctgcagctgctgaagttaaaaaagagttaaagatccaacctctagaaaaagacagcaagagtagaagctacaatgtcttggaagacaaaatcaacacagcctaccgcagttggtacctgtcctacaattacggtaaccctgagaaaggaataaggtcttggacactgctcaccacttcagatgtcacctgtggggcagagcaggtctactggtcgctccctgacatgatgcaagacccagtcaccttccgctccacaagacaagtcaacaactacccagtggtgggtgcagagcttatgcccgtcttctcaaagagtttctacaatgagcaagccgtgtactctcagcagctccgacaggccacttcgctcacgcacgtcttcaaccgcttccctgagaaccagatcctcatccgcccgccggcgcccacaattaccaccgtcagtgaaaacgttcctgctctcacagatcacgggaccctgccgttacgcagcagtatccggggagtccagcgcgtgaccgttactgacgccagacgccgcacctgtccctacgtttacaaggccctgggcatagtcgcgccgcgcgttctttcaagccgcactttctgataagcttgtcgagaagtactagaggatcataatcagccataccacatttgtagaggttttacttgctttaaaaaacctcccacacctccccctgaacctgaaacataaaatgaatgcaattgttgttgttaacttgtttattgcagcttataatggttacaaataaagcaatagcatcacaaatttcacaaataaagcatttttttcactgcattctagttgtggtttgtccaaactcatcaatgtatcttatcatgtctggatctgatcactgcttgagcctagaagatccggctgctaacaaagcccgaaaggaagctgagttggctgctgccaccgctgagcaataactatcataacccctagggtatacccatctaattggaaccagataagtgaaatctagttccaaactattttgtcatttttaattttcgtattagcttacgacgctacacccagttcccatctattttgtcactcttccctaaataatccttaaaaactccatttccacccctcccagttcccaactattttgtccgcccaca

SEQ ID NO: 62 - DNA, 4614 bp, Artificial Sequence
  Cloning vector pACEBac-ADDOMER2.0 plasmid sequence
accggttgacttgggtcaactgtcagaccaagtttactcatatatactttagattgatttaaaacttcatttttaatttaaaaggatctaggtgaagatcctttttgataatctcatgaccaaaatcccttaacgtgagttttcgttccactgagcgtcagaccccgtagaaaagatcaaaggatcttcttgagatcctttttttctgcgcgtaatctgctgcttgcaaacaaaaaaaccaccgctaccagcggtggtttgtttgccggatcaagagctaccaactctttttccgaaggtaactggcttcagcagagcgcagataccaaatactgttcttctagtgtagccgtagttaggccaccacttcaagaactctgtagcaccgcctacatacctcgctctgctaatcctgttaccagtggctgctgccagtggcgataagtcgtgtcttaccgggttggactcaagacgatagttaccggataaggcgcagcggtcgggctgaacggggggttcgtgcacacagcccagcttggagcgaacgacctacaccgaactgagatacctacagcgtgagctatgagaaagcgccacgcttcccgaagggagaaaggcggacaggtatccggtaagcggcagggtcggaacaggagagcgcacgagggagcttccagggggaaacgcctggtatctttatagtcctgtcgggtttcgccacctctgacttgagcgtcgatttttgtgatgctcgtcaggggggcggagcctatggaaaaacgccagcaacgcggcctttttacggttcctggccttttgctggccttttgctcacatgttctttcctgcgttatcccctgattgacttgggtcgctcttcctgtggatgcgcagatgccctgcgtaagcgggtgtgggcggacaataaagtcttaaactgaacaaaatagatctaaactatgacaataaagtcttaaactagacagaatagttgtaaactgaaatcagtccagttatgctgtgaaaaagcatactggacttttgttatggctaaagcaaactcttcattttctgaagtgcaaattgcccgtcgtattaaagaggggcgtggccaagggcatgtaaagactatattcgcggcgttgtgacaatttaccgaacaactccgcggccgggaagccgatctcggcttgaacgaattgttaggtggcggtacttgggtcgatatcaaagtgcatcacttcttcccgtatgcccaactttgtatagagagccactgcgggatcgtcaccgtaatctgcttgcacgtagatcacataagcaccaagcgcgttggcctcatgcttgaggagattgatgagcgcggtggcaatgccctgcctccggtgctcgccggagactgcgagatcatagatatagatctcactacgcggctgctcaaacttgggcagaacgtaagccgcgagagcgccaacaaccgcttcttggtcgaaggcagcaagcgcgatgaatgtcttactacggagcaagttcccgaggtaatcggagtccggctgatgttgggagtaggtggctacgtctccgaactcacgaccgaaaagatcaagagcagcccgcatggatttgacttggtcagggccgagcctacatgtgcgaatgatgcccatacttgagccacctaactttgttttagggcgactgccctgctgcgtaacatcgttgctgctgcgtaacatcgttgctgctccataacatcaaacatcgacccacggcgtaacgcgcttgctgcttggatgcccgaggcatagactgtacaaaaaaacagtcataacaagccatgaaaaccgccactgcgccgttaccaccgctgcgttcggtcaaggttctggaccagttgcgtgagcgcatacgctacttgcattacagtttacgaaccgaacaggcttatgtcaactgggttcgtgccttcatccgtttccacggtgtgcgtcacccggcaaccttgggcagcagcgaagtcgccataacttcgtatagcatacattatacgaagttatctgtaactataacggtcctaaggtagcgagtttaaacactagtatcgattcgcgacctactccggaatattaatagatcatggagataattaaaatgataaccatctcgcaaataaataagtattttactgttttcgtaacagttttgtaataaaaaaacctataaatattccggattattcataccgtcccaccatcgggcgcggatccatgaggagacgagccgtgctaggcggagcggtggtgtatccggagggtcctcctccttcttacgagagcgtgatgcagcaacaggcggcgatgatacagcccccactggaggctcccttcgtacccccacggtacctggcgcctacggaagggagaaacagcattcgttactcggagctgtcgcccctgtacgataccaccaagttgtatctggtggacaacaagtcggcggacatcgcctccctgaactatcagaacgaccacagcaacttcctgaccacggtggtgcagaacaatgactttacccccacggaggctagcacccagaccatcaactttgacgagcggtcgcgatggggcggtcagctgaagaccatcatgcacaccaacatgcccaacgtgaacgagtacatgttcagcaacaagttcaaggcgagggtgatggtgtccagaaaagctcctgaaggtgaattcgttacagtcaatgacggtccggtcaatgacacctatgatcataaagaggatatcttgaagtatgagtggtttgagttcattttaccagaaggcaacttttcagccaccatgacgatcgacctgatgaacaatgccatcattgacaactacctggaaattggcagacagaatggagtgctggaaagtgacattggtgttaagtttgacactagaaatttcaggctcgggtgggaccccgaaactaagttgattatgccaggtgtctacacttatgaggcattccatcctgacattgtattgctgcctggttgcggggtagactttactgaaagccgacttagcaacttgcttggcatcaggaagagacatccattccaggagggtttcaaaatcatgtatgaagatcttgaagggggtaatattcctgcccttttggatgtcactgcctatgaggaaagcaaaaaggataccactactgcgcgcgaaacaaccacactggctgttgcagaggaaactagtgaagatgtcgacgatgatataactagaggagatacctatataactgagctcgaaaaacaaaaacgtgaagctgctgctgctgaagtttctagaaaaaaagagttaaagatccaacctctggaaaaagacagcaagagtagaagctacaatgtcttggaagacaaaatcaacacagcctaccgcagttggtatctgtcctacaattacggtaaccctgagaaaggaataaggtcttggacactgctcaccacttcagatgtcacctgtggggcagagcaggtctactggtcgctccctgacatgatgcaagacccagtcaccttccgctccacaagacaagtcaacaactacccagtggtgggtgcagagcttatgcccgtcttctcaaagagtttctacaatgagcaagccgtgtactctcagcagctccgacaggccacttcgctcacgcacgtcttcaaccgcttccctgagaaccagatcctcatccgcccgccggcacccacaattaccaccgtcagtgaaaacgttcctgctctcacagatcacgggaccctgccgttacgcagcagtatccggggagtccagcgcgtgaccgttactgacgccagacgccgcacctgtccctacgtttacaaggccctgggcatagtcgcgccgcgcgttctttcaagccgcactttctgataagcttccatcaactttgacgagcggtcgcgatggggcggtcagctgaagaccatcatgcacaccaacatgcccaacgtgaacgagtacatgttcagcaacaagttcaaggcgagggagcttgtcgagaagtactagaggatcataatcagccataccacatttgtagaggttttacttgctttaaaaaacctcccacacctccccctgaacctgaaacataaaatgaatgcaattgttgttgttaacttgtttattgcagcttataatggttacaaataaagcaatagcatcacaaatttcacaaataaagcatttttttcactgcattctagttgtggtttgtccaaactcatcaatgtatcttatcatgtctggatctgatcactgcttgagcctagaagatccggctgctaacaaagcccgaaaggaagctgagttggctgctgccaccgctgagcaataactatcataacccctagggtatacccatctaattggaaccagataagtgaaatctagttccaaactattttgtcatttttaattttcgtattagcttacgacgctacacccagttcccatctattttgtcactcttccctaaataatccttaaaaactccatttccacccctcccagttcccaactattttgtccgcccaca

SEQ ID NO: 63 - DNA, 1683 bp, Artificial Sequence
  ADDomere 1 engineered penton base protomer nucleic acid sequence ready for insertion of heterologous polypeptides
atgaggagacgagccgtgctaggcggagcggtggtgtatccggagggtcctcctccttcttacgagagcgtgatgcagcaacaggcggcgatgatacagcccccactggaggctcccttcgtacccccacggtacctggcgcctacggaagggagaaacagcattcgttactcggagctgtcgcccctgtacgataccaccaagttgtatctggtggacaacaagtcggcggacatcgcctccctgaactatcagaacgaccacagcaacttcctgaccacggtggtgcagaacaatgactttacccccacggaggctagcacccagaccatcaactttgacgagcggtcgcgatggggcggtcagctgaagaccatcatgcacaccaacatgcccaacgtgaacgagtacatgttcagcaacaagttcaaggcgagggtgatggtgtccagaaaagctcctgaaggtgaattcgttacagtcaatgacggtccggtcaatgacacctatgatcataaagaggatatcttgaagtatgagtggtttgagttcattttaccagaaggcaacttttcagccaccatgacgatcgacctgatgaacaatgccatcattgacaactacctggaaattggcagacagaatggagtgctggaaagtgacattggtgttaagtttgacactagaaatttcaggctcgggtgggaccccgaaactaagttgattatgccaggtgtctacacttatgaggcattccatcctgacattgtattgctgcctggttgcggggtagactttactgaaagccgacttagcaacttgcttggcatcaggaagagacatccattccaggagggtttcaaaatcatgtatgaagatcttgaagggggtaatattcctgcccttttggatgtcactgcctatgaggaaagcaaaaaggataccactactgcgcgcgaaacaaccacactggctgttgcagaggaaactagtgaagatgtcgacgatgatataactagaggagatacctatataactgagctcgaaaaacaaaaacgtgaagctgctgctgctgaagtttctagaaaaaaagagttaaagatccaacctctggaaaaagacagcaagagtagaagctacaatgtcttggaagacaaaatcaacacagcctaccgcagttggtatctgtcctacaattacggtaaccctgagaaaggaataaggtcttggacactgctcaccacttcagatgtcacctgtggggcagagcaggtctactggtcgctccctgacatgatgcaagacccagtcaccttccgctccacaagacaagtcaacaactacccagtggtgggtgcagagcttatgcccgtcttctcaaagagtttctacaatgagcaagccgtgtactctcagcagctccgacaggccacttcgctcacgcacgtcttcaaccgcttccctgagaaccagatcctcatccgcccgccggcacccacaattaccaccgtcagtgaaaacgttcctgctctcacagatcacgggaccctgccgttacgcagcagtatccggggagtccagcgcgtgaccgttactgacgccagacgccgcacctgtccctacgtttacaaggccctgggcatagtcgcgccgcgcgttctttcaagccgcactttctgataa

SEQ ID NO: 64 - protein, 559 aa, Artificial Sequence
  ADDomere 1.0 protein sequence ready for insertion of heterologous polypeptides
MRRRAVLGGAVVYPEGPPPSYESVMQQQAAMIQPPLEAPFVPPRYLAPTEGRNSIRYSELSPLYDTTKLYLVDNKSADIASLNYQNDHSNFLTTVVQNNDFTPTEASTQTINFDERSRWGGQLKTIMHTNMPNVNEYMFSNKFKARVMVSRKAPEGEFVTVNDGPVNDTYDHKEDILKYEWFEFILPEGNFSATMTIDLMNNAIIDNYLEIGRQNGVLESDIGVKFDTRNFRLGWDPETKLIMPGVYTYEAFHPDIVLLPGCGVDFTESRLSNLLGIRKRHPFQEGFKIMYEDLEGGNIPALLDVTAYEESKKDTTTARETTTLAVAEETSEDVDDDITRGDTYITELEKQKREAAAAEVSRKKELKIQPLEKDSKSRSYNVLEDKINTAYRSWYLSYNYGNPEKGIRSWTLLTTSDVTCGAEQVYWSLPDMMQDPVTFRSTRQVNNYPVVGAELMPVFSKSFYNEQAVYSQQLRQATSLTHVFNRFPENQILIRPPAPTITTVSENVPALTDHGTLPLRSSIRGVQRVTVTDARRRTCPYVYKALGIVAPRVLSSRTF

SEQ ID NO: 65 - protein, 559 aa, Artificial Sequence
  ADDomere 2.0 protein sequence with coupling residues at position 51 and 54
MRRRAVLGGAVVYPEGPPPSYESVMQQQAAMIQPPLEAPFVPPRYLAPTECRNCIRYSELSPLYDTTKLYLVDNKSADIASLNYQNDHSNFLTTVVQNNDFTPTEASTQTINFDERSRWGGQLKTIMHTNMPNVNEYMFSNKFKARVMVSRKAPEGEFVTVNDGPVNDTYDHKEDILKYEWFEFILPEGNFSATMTIDLMNNAIIDNYLEIGRQNGVLESDIGVKFDTRNFRLGWDPETKLIMPGVYTYEAFHPDIVLLPGCGVDFTESRLSNLLGIRKRHPFQEGFKIMYEDLEGGNIPALLDVTAYEESKKDTTTARETTTLAVAEETSEDVDDDITRGDTYITELEKQKREAAAAEVSRKKELKIQPLEKDSKSRSYNVLEDKINTAYRSWYLSYNYGNPEKGIRSWTLLTTSDVTCGAEQVYWSLPDMMQDPVTFRSTRQVNNYPVVGAELMPVFSKSFYNEQAVYSQQLRQATSLTHVFNRFPENQILIRPPAPTITTVSENVPALTDHGTLPLRSSIRGVQRVTVTDARRRTCPYVYKALGIVAPRVLSSRTF

SEQ ID NO: 66 - protein, 559 aa, Artificial Sequence
  ADDomere 2.0 protein sequence with coupling residues at position 51 and 114
MRRRAVLGGAVVYPEGPPPSYESVMQQQAAMIQPPLEAPFVPPRYLAPTEGRNCIRYSELSPLYDTTKLYLVDNKSADIASLNYQNDHSNFLTTVVQNNDFTPTEASTQTINFCERSRWGGQLKTIMHTNMPNVNEYMFSNKFKARVMVSRKAPEGEFVTVNDGPVNDTYDHKEDILKYEWFEFILPEGNFSATMTIDLMNNAIIDNYLEIGRQNGVLESDIGVKFDTRNFRLGWDPETKLIMPGVYTYEAFHPDIVLLPGCGVDFTESRLSNLLGIRKRHPFQEGFKIMYEDLEGGNIPALLDVTAYEESKKDTTTARETTTLAVAEETSEDVDDDITRGDTYITELEKQKREAAAAEVSRKKELKIQPLEKDSKSRSYNVLEDKINTAYRSWYLSYNYGNPEKGIRSWTLLTTSDVTCGAEQVYWSLPDMMQDPVTFRSTRQVNNYPVVGAELMPVFSKSFYNEQAVYSQQLRQATSLTHVFNRFPENQILIRPPAPTITTVSENVPALTDHGTLPLRSSIRGVQRVTVTDARRRTCPYVYKALGIVAPRVLSSRTF

SEQ ID NO: 67 - protein, 559 aa, Artificial Sequence
  ADDomere 2.0 protein sequence with coupling residues at position 51 and 541
MRRRAVLGGAVVYPEGPPPSYESVMQQQAAMIQPPLEAPFVPPRYLAPTEGRCSIRYSELSPLYDTTKLYLVDNKSADIASLNYQNDHSNFLTTVVQNNDFTPTEASTQTINFDERSRWGGQLKTIMHTNMPNVNEYMFSNKFKARVMVSRKAPEGEFVTVNDGPVNDTYDHKEDILKYEWFEFILPEGNFSATMTIDLMNNAIIDNYLEIGRQNGVLESDIGVKFDTRNFRLGWDPETKLIMPGVYTYEAFHPDIVLLPGCGVDFTESRLSNLLGIRKRHPFQEGFKIMYEDLEGGNIPALLDVTAYEESKKDTTTARETTTLAVAEETSEDVDDDITRGDTYITELEKQKREAAAAEVSRKKELKIQPLEKDSKSRSYNVLEDKINTAYRSWYLSYNYGNPEKGIRSWTLLTTSDVTCGAEQVYWSLPDMMQDPVTFRSTRQVNNYPVVGAELMPVFSKSFYNEQAVYSQQLRQATSLTHVFNRFPENQILIRPPAPTITTVSENVPALTDHGTLPLRSSIRGVQRVTVTDARRRTCPCVYKALGIVAPRVLSSRTF

SEQ ID NO: 68 - protein, 10 aa, Artificial Sequence
  Consenus sequence of penton base protomer in the STICKER binding cleft
  MISC_FEATURE (4)..(4): Xaa is selected from the group consisting of Y and F
  MISC_FEATURE (6)..(6): Xaa is selected from the group consisting of D, E and a coupling residue, preferably Cys
  MISC_FEATURE (7)..(7): Xaa is selected from the group consisting of L, Q and a coupling residue, preferably Cys
KSFXNXXAVY

SEQ ID NO: 69 - protein, 12 aa, Artificial Sequence
  STICKER N-terminal fragment of fibre comprising acoupling residue
  MISC_FEATURE (1)..(1): Xaa is selected from the group consisting of S, D and T
  MISC_FEATURE (9)..(9): Xaa is selected from the group consisting of E, D and G
  MISC_FEATURE (10)..(10): Xaa is in each case independently any amino acid, preferably those naturally occurring in fibre proteins at this or these positions
  MISC_FEATURE (11)..(11): Xaa is a coupling residue, preferably Cys
  misc_feature (12)..(12): Xaa can be any naturally occurring amino acid
XFNPVYPYXXNX

SEQ ID NO: 70 - protein, 9 aa, Artificial Sequence
  STICKER N-terminal fragment of fibre comprising a coupling residue
  MISC_FEATURE (1)..(1): Xaa is a coupling residue, preferably Cys
  MISC_FEATURE (9)..(9): Xaa is selected from the group consisting of E, D and G
XFNPVYPYX

SEQ ID NO: 71 - DNA, 4692 bp, Artificial Sequence
  pACEBac-ADDomer2.0TevChik plasmid sequence
accggttgacttgggtcaactgtcagaccaagtttactcatatatactttagattgatttaaaacttcatttttaatttaaaaggatctaggtgaagatcctttttgataatctcatgaccaaaatcccttaacgtgagttttcgttccactgagcgtcagaccccgtagaaaagatcaaaggatcttcttgagatcctttttttctgcgcgtaatctgctgcttgcaaacaaaaaaaccaccgctaccagcggtggtttgtttgccggatcaagagctaccaactctttttccgaaggtaactggcttcagcagagcgcagataccaaatactgttcttctagtgtagccgtagttaggccaccacttcaagaactctgtagcaccgcctacatacctcgctctgctaatcctgttaccagtggctgctgccagtggcgataagtcgtgtcttaccgggttggactcaagacgatagttaccggataaggcgcagcggtcgggctgaacggggggttcgtgcacacagcccagcttggagcgaacgacctacaccgaactgagatacctacagcgtgagctatgagaaagcgccacgcttcccgaagggagaaaggcggacaggtatccggtaagcggcagggtcggaacaggagagcgcacgagggagcttccagggggaaacgcctggtatctttatagtcctgtcgggtttcgccacctctgacttgagcgtcgatttttgtgatgctcgtcaggggggcggagcctatggaaaaacgccagcaacgcggcctttttacggttcctggccttttgctggccttttgctcacatgttctttcctgcgttatcccctgattgacttgggtcgctcttcctgtggatgcgcagatgccctgcgtaagcgggtgtgggcggacaataaagtcttaaactgaacaaaatagatctaaactatgacaataaagtcttaaactagacagaatagttgtaaactgaaatcagtccagttatgctgtgaaaaagcatactggacttttgttatggctaaagcaaactcttcattttctgaagtgcaaattgcccgtcgtattaaagaggggcgtggccaagggcatgtaaagactatattcgcggcgttgtgacaatttaccgaacaactccgcggccgggaagccgatctcggcttgaacgaattgttaggtggcggtacttgggtcgatatcaaagtgcatcacttcttcccgtatgcccaactttgtatagagagccactgcgggatcgtcaccgtaatctgcttgcacgtagatcacataagcaccaagcgcgttggcctcatgcttgaggagattgatgagcgcggtggcaatgccctgcctccggtgctcgccggagactgcgagatcatagatatagatctcactacgcggctgctcaaacttgggcagaacgtaagccgcgagagcgccaacaaccgcttcttggtcgaaggcagcaagcgcgatgaatgtcttactacggagcaagttcccgaggtaatcggagtccggctgatgttgggagtaggtggctacgtctccgaactcacgaccgaaaagatcaagagcagcccgcatggatttgacttggtcagggccgagcctacatgtgcgaatgatgcccatacttgagccacctaactttgttttagggcgactgccctgctgcgtaacatcgttgctgctgcgtaacatcgttgctgctccataacatcaaacatcgacccacggcgtaacgcgcttgctgcttggatgcccgaggcatagactgtacaaaaaaacagtcataacaagccatgaaaaccgccactgcgccgttaccaccgctgcgttcggtcaaggttctggaccagttgcgtgagcgcatacgctacttgcattacagtttacgaaccgaacaggcttatgtcaactgggttcgtgccttcatccgtttccacggtgtgcgtcacccggcaaccttgggcagcagcgaagtcgccataacttcgtatagcatacattatacgaagttatctgtaactataacggtcctaaggtagcgagtttaaacactagtatcgattcgcgacctactccggaatattaatagatcatggagataattaaaatgataaccatctcgcaaataaataagtattttactgttttcgtaacagttttgtaataaaaaaacctataaatattccggattattcataccgtcccaccatcgggcgcggatccatgaggagacgagccgtgctaggcggagcggtggtgtatccggagggtcctcctccttcttacgagagcgtgatgcagcaacaggcggcgatgatacagcccccactggaggctcccttcgtacccccacggtacctggcgcctacggaagggagaaacagcattcgttactcggagctgtcgcccctgtacgataccaccaagttgtatctggtggacaacaagtcggcggacatcgcctccctgaactatcagaacgaccacagcaacttcctgaccacggtggtgcagaacaatgactttacccccacggaggctagcacccagaccatcaactttgacgagcggtcgcgatggggcggtcagctgaagaccatcatgcacaccaacatgcccaacgtgaacgagtacatgttcagcaacaagttcaaggcgagggtgatggtgtccagaaaagctcctgaaggtgaattcggcagcggtggcgaaaacctgtattttcagagcaccaaagataactttaacgtgtataaagcgacccgcccgtatctggcgcatggtggcagcggtccggtcaatgacacctatgatcataaagaggatatcttgaagtatgagtggtttgagttcattttaccagaaggcaacttttcagccaccatgacgatcgacctgatgaacaatgccatcattgacaactacctggaaattggcagacagaatggagtgctggaaagtgacattggtgttaagtttgacactagaaatttcaggctcgggtgggaccccgaaactaagttgattatgccaggtgtctacacttatgaggcattccatcctgacattgtattgctgcctggttgcggggtagactttactgaaagccgacttagcaacttgcttggcatcaggaagagacatccattccaggagggtttcaaaatcatgtatgaagatcttgaagggggtaatattcctgcccttttggatgtcactgcctatgaggaaagcaaaaaggataccactactgcgcgcgaaacaaccacactggctgttgcagaggaaactagtgaagatgtcgacgatgatataactagaggagatacctatataactgagctcgaaaaacaaaaacgtgaagctgctgctgctgaagtttctagaaaaaaagagttaaagatccaacctctggaaaaagacagcaagagtagaagctacaatgtcttggaagacaaaatcaacacagcctaccgcagttggtatctgtcctacaattacggtaaccctgagaaaggaataaggtcttggacactgctcaccacttcagatgtcacctgtggggcagagcaggtctactggtcgctccctgacatgatgcaagacccagtcaccttccgctccacaagacaagtcaacaactacccagtggtgggtgcagagcttatgcccgtcttctcaaagagtttctacaatgagcaagccgtgtactctcagcagctccgacaggccacttcgctcacgcacgtcttcaaccgcttccctgagaaccagatcctcatccgcccgccggcacccacaattaccaccgtcagtgaaaacgttcctgctctcacagatcacgggaccctgccgttacgcagcagtatccggggagtccagcgcgtgaccgttactgacgccagacgccgcacctgtccctacgtttacaaggccctgggcatagtcgcgccgcgcgttctttcaagccgcactttctgataagcttccatcaactttgacgagcggtcgcgatggggcggtcagctgaagaccatcatgcacaccaacatgcccaacgtgaacgagtacatgttcagcaacaagttcaaggcgagggagcttgtcgagaagtactagaggatcataatcagccataccacatttgtagaggttttacttgctttaaaaaacctcccacacctccccctgaacctgaaacataaaatgaatgcaattgttgttgttaacttgtttattgcagcttataatggttacaaataaagcaatagcatcacaaatttcacaaataaagcatttttttcactgcattctagttgtggtttgtccaaactcatcaatgtatcttatcatgtctggatctgatcactgcttgagcctagaagatccggctgctaacaaagcccgaaaggaagctgagttggctgctgccaccgctgagcaataactatcataacccctagggtatacccatctaattggaaccagataagtgaaatctagttccaaactattttgtcatttttaattttcgtattagcttacgacgctacacccagttcccatctattttgtcactcttccctaaataatccttaaaaactccatttccacccctcccagttcccaactattttgtccgcccaca

SEQ ID NO: 72 - DNA, 4788 bp, Artificial Sequence
  pACEBac-ADDOmer2.0-[TevCHIK]2 plasmid sequence
accggttgacttgggtcaactgtcagaccaagtttactcatatatactttagattgatttaaaacttcatttttaatttaaaaggatctaggtgaagatcctttttgataatctcatgaccaaaatcccttaacgtgagttttcgttccactgagcgtcagaccccgtagaaaagatcaaaggatcttcttgagatcctttttttctgcgcgtaatctgctgcttgcaaacaaaaaaaccaccgctaccagcggtggtttgtttgccggatcaagagctaccaactctttttccgaaggtaactggcttcagcagagcgcagataccaaatactgttcttctagtgtagccgtagttaggccaccacttcaagaactctgtagcaccgcctacatacctcgctctgctaatcctgttaccagtggctgctgccagtggcgataagtcgtgtcttaccgggttggactcaagacgatagttaccggataaggcgcagcggtcgggctgaacggggggttcgtgcacacagcccagcttggagcgaacgacctacaccgaactgagatacctacagcgtgagctatgagaaagcgccacgcttcccgaagggagaaaggcggacaggtatccggtaagcggcagggtcggaacaggagagcgcacgagggagcttccagggggaaacgcctggtatctttatagtcctgtcgggtttcgccacctctgacttgagcgtcgatttttgtgatgctcgtcaggggggcggagcctatggaaaaacgccagcaacgcggcctttttacggttcctggccttttgctggccttttgctcacatgttctttcctgcgttatcccctgattgacttgggtcgctcttcctgtggatgcgcagatgccctgcgtaagcgggtgtgggcggacaataaagtcttaaactgaacaaaatagatctaaactatgacaataaagtcttaaactagacagaatagttgtaaactgaaatcagtccagttatgctgtgaaaaagcatactggacttttgttatggctaaagcaaactcttcattttctgaagtgcaaattgcccgtcgtattaaagaggggcgtggccaagggcatgtaaagactatattcgcggcgttgtgacaatttaccgaacaactccgcggccgggaagccgatctcggcttgaacgaattgttaggtggcggtacttgggtcgatatcaaagtgcatcacttcttcccgtatgcccaactttgtatagagagccactgcgggatcgtcaccgtaatctgcttgcacgtagatcacataagcaccaagcgcgttggcctcatgcttgaggagattgatgagcgcggtggcaatgccctgcctccggtgctcgccggagactgcgagatcatagatatagatctcactacgcggctgctcaaacttgggcagaacgtaagccgcgagagcgccaacaaccgcttcttggtcgaaggcagcaagcgcgatgaatgtcttactacggagcaagttcccgaggtaatcggagtccggctgatgttgggagtaggtggctacgtctccgaactcacgaccgaaaagatcaagagcagcccgcatggatttgacttggtcagggccgagcctacatgtgcgaatgatgcccatacttgagccacctaactttgttttagggcgactgccctgctgcgtaacatcgttgctgctgcgtaacatcgttgctgctccataacatcaaacatcgacccacggcgtaacgcgcttgctgcttggatgcccgaggcatagactgtacaaaaaaacagtcataacaagccatgaaaaccgccactgcgccgttaccaccgctgcgttcggtcaaggttctggaccagttgcgtgagcgcatacgctacttgcattacagtttacgaaccgaacaggcttatgtcaactgggttcgtgccttcatccgtttccacggtgtgcgtcacccggcaaccttgggcagcagcgaagtcgccataacttcgtatagcatacattatacgaagttatctgtaactataacggtcctaaggtagcgagtttaaacactagtatcgattcgcgacctactccggaatattaatagatcatggagataattaaaatgataaccatctcgcaaataaataagtattttactgttttcgtaacagttttgtaataaaaaaacctataaatattccggattattcataccgtcccaccatcgggcgcggatccatgaggagacgagccgtgctaggcggagcggtggtgtatccggagggtcctcctccttcttacgagagcgtgatgcagcaacaggcggcgatgatacagcccccactggaggctcccttcgtacccccacggtacctggcgcctacggaagggagaaacagcattcgttactcggagctgtcgcccctgtacgataccaccaagttgtatctggtggacaacaagtcggcggacatcgcctccctgaactatcagaacgaccacagcaacttcctgaccacggtggtgcagaacaatgactttacccccacggaggctagcacccagaccatcaactttgacgagcggtcgcgatggggcggtcagctgaagaccatcatgcacaccaacatgcccaacgtgaacgagtacatgttcagcaacaagttcaaggcgagggtgatggtgtccagaaaagctcctgaaggtgaattcggcagcggtggcgaaaacctgtattttcagagcaccaaagataactttaacgtgtataaagcgacccgcccgtatctggcgcatggtggcagcggtccggtcaatgacacctatgatcataaagaggatatcttgaagtatgagtggtttgagttcattttaccagaaggcaacttttcagccaccatgacgatcgacctgatgaacaatgccatcattgacaactacctggaaattggcagacagaatggagtgctggaaagtgacattggtgttaagtttgacactagaaatttcaggctcgggtgggaccccgaaactaagttgattatgccaggtgtctacacttatgaggcattccatcctgacattgtattgctgcctggttgcggggtagactttactgaaagccgacttagcaacttgcttggcatcaggaagagacatccattccaggagggtttcaaaatcatgtatgaagatcttgaagggggtaatattcctgcccttttggatgtcactgcctatgaggaaagcaaaaaggataccactactgcgcgcgaaacaaccacactggctgttgcagaggaaactagtgaagatgtcgacgatgatataactagaggagatacctatataactgagctcggcagcggtggcgaaaacctgtattttcagagcaccaaagataactttaacgtgtataaagcgacccgcccgtatctggcgcatggtggcagcggtgaaaaacaaaaacgtgaagctgctgctgctgaagtttctagaaaaaaagagttaaagatccaacctctggaaaaagacagcaagagtagaagctacaatgtcttggaagacaaaatcaacacagcctaccgcagttggtatctgtcctacaattacggtaaccctgagaaaggaataaggtcttggacactgctcaccacttcagatgtcacctgtggggcagagcaggtctactggtcgctccctgacatgatgcaagacccagtcaccttccgctccacaagacaagtcaacaactacccagtggtgggtgcagagcttatgcccgtcttctcaaagagtttctacaatgagcaagccgtgtactctcagcagctccgacaggccacttcgctcacgcacgtcttcaaccgcttccctgagaaccagatcctcatccgcccgccggcacccacaattaccaccgtcagtgaaaacgttcctgctctcacagatcacgggaccctgccgttacgcagcagtatccggggagtccagcgcgtgaccgttactgacgccagacgccgcacctgtccctacgtttacaaggccctgggcatagtcgcgccgcgcgttctttcaagccgcactttctgataagcttccatcaactttgacgagcggtcgcgatggggcggtcagctgaagaccatcatgcacaccaacatgcccaacgtgaacgagtacatgttcagcaacaagttcaaggcgagggagcttgtcgagaagtactagaggatcataatcagccataccacatttgtagaggttttacttgctttaaaaaacctcccacacctccccctgaacctgaaacataaaatgaatgcaattgttgttgttaacttgtttattgcagcttataatggttacaaataaagcaatagcatcacaaatttcacaaataaagcatttttttcactgcattctagttgtggtttgtccaaactcatcaatgtatcttatcatgtctggatctgatcactgcttgagcctagaagatccggctgctaacaaagcccgaaaggaagctgagttggctgctgccaccgctgagcaataactatcataacccctagggtatacccatctaattggaaccagataagtgaaatctagttccaaactattttgtcatttttaattttcgtattagcttacgacgctacacccagttcccatctattttgtcactcttccctaaataatccttaaaaactccatttccacccctcccagttcccaactattttgtccgcccaca

SEQ ID NO: 73 - protein, 6 aa, Artificial Sequence
  Consenus sequence of penton base protomer in the STICKER binding cleft
  MISC_FEATURE (1)..(1): Xaa is a coupling residue, preferably C, D, E, and K, most preferably C
  MISC_FEATURE (2)..(2): Xaa is any amino acid, is preferably selected from the group consisting of D, E, G, K, N, or S, more preferably S or N
XXRSYN

SEQ ID NO: 74 - protein, 20 aa, Artificial Sequence
  STICKER N-terminal fragment of fibre comprising acoupling residue
  MISC_FEATURE (9)..(9): Xaa is a coupling residue selected from the group comprising K, C, D or E, preferably C
  MISC_FEATURE (16)..(16): Xaa is selected from the group consisting of E, D and G, is preferably E or D, and is more preferably E
  misc_feature (17)..(17): Xaa can be any naturally occurring amino acid
AKRARLSTXFNPVYPYXDES

SEQ ID NO: 75 - protein, 20 aa, Artificial Sequence
  STICKER N-terminal fragment of fibre comprising acoupling residue
AKRARLSTCFNPVYPYEDES

SEQ ID NO: 76 - protein, 20 aa, Artificial Sequence
  STICKER N-terminal fragment of fibre comprising acoupling residue
  MISC_FEATURE (9)..(9): Xaa is selected from the group consisting of S, D and T, preferably S or D, and is more preferably S
  MISC_FEATURE (16)..(16): Xaa is selected from the group consisting of E, D and G, is preferably E or D, and is more preferably E
  misc_feature (17)..(17): Xaa can be any naturally occurring amino acid
  MISC_FEATURE (20)..(20): Xaa is a coupling residue, preferably C, D, E, and K, most preferably C
AKRARLSTXFNPVYPYXDEX

SEQ ID NO: 77 - protein, 20 aa, Artificial Sequence
  STICKER N-terminal fragment of fibre comprising acoupling residue
AKRARLSTSFNPVYPYEDEC

SEQ ID NO: 78 - protein, 32 aa, Artificial Sequence
  Chikunguny epitope construct inserted into penton base protomer
GSGGENLYFQSTKDNFNVYKATRPYLAHGGSG